European Patent Application EP 4 134 084 A2, published February 15, 2023. Title: Tissue-specifically expressed circular RNA molecule and application thereof. Applicant: Suzhou Curemed Biomedical Technology Co. Ltd. The sequence listing filed with the application follows.

SEQUENCE LISTING (97 sequences)

SEQ ID NO: 1 - RNA, 119 nt, synthetic construct
  misc_feature 1..119: note = sequence of 3'UTR
  source 1..119: mol_type = other RNA
tgataataggctggagcctcggtggccatgcttcttgccccttgggcctccccccagcccctcctccccttcctgcacccgtacccccgtggtctttgaataaagtctgagtgggcggc

SEQ ID NO: 2 - RNA, 22 nt, Homo sapiens
  source 1..22: mol_type = other RNA
caaacaccattgtcacactcca

SEQ ID NO: 3 - RNA, 21 nt, Homo sapiens
  source 1..21: mol_type = other RNA
ccaagttctgtcatgcactga

SEQ ID NO: 4 - RNA, 22 nt, Homo sapiens
  source 1..22: mol_type = other RNA
agtcggagtgtctcagaacttt

SEQ ID NO: 5 - RNA, 22 nt, Homo sapiens
  source 1..22: mol_type = other RNA
tccacatggagttgctgttaca

SEQ ID NO: 6 - RNA, 22 nt, Homo sapiens
  source 1..22: mol_type = other RNA
taaccaatgtgcagactactgt

SEQ ID NO: 7 - RNA, 21 nt, Homo sapiens
  source 1..21: mol_type = other RNA
gtctgtcaattcataggtcat

SEQ ID NO: 8 - RNA, 23 nt, Homo sapiens
  source 1..23: mol_type = other RNA
ctatctgcactagatgcacctta

SEQ ID NO: 9 - RNA, 23 nt, Homo sapiens
  source 1..23: mol_type = other RNA
ctacctgcactataagcacttta

SEQ ID NO: 10 - RNA, 22 nt, Homo sapiens
  source 1..22: mol_type = other RNA
ctgttcctgctgaactgagcca

SEQ ID NO: 11 - RNA, 22 nt, Homo sapiens
  source 1..22: mol_type = other RNA
agctgagtgtaggatgtttaca

SEQ ID NO: 12 - RNA, 23 nt, Homo sapiens
  source 1..23: mol_type = other RNA
gctgagagtgtaggatgtttaca

SEQ ID NO: 13 - RNA, 22 nt, Homo sapiens
  source 1..22: mol_type = other RNA
tgcaacttagtaatgtgcaata

SEQ ID NO: 14 - RNA, 22 nt, Homo sapiens
  source 1..22: mol_type = other RNA
ccatctttaccagacagtgtta

SEQ ID NO: 15 - RNA, 21 nt, Homo sapiens
  source 1..21: mol_type = other RNA
ggctgtcaattcataggtcag

SEQ ID NO: 16 - RNA, 22 nt, Homo sapiens
  source 1..22: mol_type = other RNA
tcatctcgcccgcaaagaccca

SEQ ID NO: 17 - RNA, 22 nt, Homo sapiens
  source 1..22: mol_type = other RNA
tccacatggagttgctgttaca

SEQ ID NO: 18 - RNA, 22 nt, Homo sapiens
  source 1..22: mol_type = other RNA
tcatcattaccaggcagtatta

SEQ ID NO: 19 - RNA, 22 nt, Homo sapiens
  source 1..22: mol_type = other RNA
aggcataggatgacaaagggaa

SEQ ID NO: 20 - RNA, 23 nt, Homo sapiens
  source 1..23: mol_type = other RNA
ctatctgcactagatgcacctta

SEQ ID NO: 21 - RNA, 23 nt, Homo sapiens
  source 1..23: mol_type = other RNA
tcagttttgcatagatttgcaca

SEQ ID NO: 22 - RNA, 23 nt, Homo sapiens
  source 1..23: mol_type = other RNA
ctacctgcactataagcacttta

SEQ ID NO: 23 - RNA, 22 nt, Homo sapiens
  source 1..22: mol_type = other RNA
ctgttcctgctgaactgagcca

SEQ ID NO: 24 - RNA, 22 nt, Homo sapiens
  source 1..22: mol_type = other RNA
tgcaacttagtaatgtgcaata

SEQ ID NO: 25 - RNA, 22 nt, Homo sapiens
  source 1..22: mol_type = other RNA
cgcattattactcacggtacga

SEQ ID NO: 26 - RNA, 22 nt, Homo sapiens
  source 1..22: mol_type = other RNA
cagctggttgaaggggaccaaa

SEQ ID NO: 27 - RNA, 22 nt, Homo sapiens
  source 1..22: mol_type = other RNA
ccatctttaccagacagtgtta

SEQ ID NO: 28 - RNA, 22 nt, Homo sapiens
  source 1..22: mol_type = other RNA
tcatctcgcccgcaaagaccca

SEQ ID NO: 29 - RNA, 22 nt, Homo sapiens
  source 1..22: mol_type = other RNA
tcatcattaccaggcagtatta

SEQ ID NO: 30 - RNA, 23 nt, Homo sapiens
  source 1..23: mol_type = other RNA
actcaccgacagcgttgaatgtt

SEQ ID NO: 31 - RNA, 22 nt, Homo sapiens
  source 1..22: mol_type = other RNA
atacatacttctttacattcca

SEQ ID NO: 32 - RNA, 22 nt, Homo sapiens
  source 1..22: mol_type = other RNA
cagctggttgaaggggaccaaa

SEQ ID NO: 33 - RNA, 21 nt, Homo sapiens
  source 1..21: mol_type = other RNA
gagctacagtgcttcatctca

SEQ ID NO: 34 - RNA, 23 nt, Homo sapiens
  source 1..23: mol_type = other RNA
gggagtgaagacacggagccaga

SEQ ID NO: 35 - RNA, 22 nt, Homo sapiens
  source 1..22: mol_type = other RNA
ccacacacttccttacattcca

SEQ ID NO: 36 - RNA, 22 nt, Homo sapiens
  source 1..22: mol_type = other RNA
gtataacccgggccaaaagctc

SEQ ID NO: 37 - RNA, 24 nt, Homo sapiens
  source 1..24: mol_type = other RNA
aacaacaaaatcactagtcttcca

SEQ ID NO: 38 - RNA, 23 nt, Homo sapiens
  source 1..23: mol_type = other RNA
tcatacagctagataaccaaaga

SEQ ID NO: 39 - RNA, 22 nt, Homo sapiens
  source 1..22: mol_type = other RNA
ttggcattcaccgcgtgcctta

SEQ ID NO: 40 - RNA, 24 nt, Homo sapiens
  source 1..24: mol_type = other RNA
tcacaggttaaagggtctcaggga

SEQ ID NO: 41 - RNA, 21 nt, Homo sapiens
  source 1..21: mol_type = other RNA
aaagagaccggttcactgtga

SEQ ID NO: 42 - RNA, 22 nt, Homo sapiens
  source 1..22: mol_type = other RNA
cgaccatggctgtagactgtta

SEQ ID NO: 43 - RNA, 23 nt, Homo sapiens
  source 1..23: mol_type = other RNA
tcacataggaataaaaagccata

SEQ ID NO: 44 - RNA, 23 nt, Homo sapiens
  source 1..23: mol_type = other RNA
ctacgcgtattcttaagcaataa

SEQ ID NO: 45 - RNA, 23 nt, Homo sapiens
  source 1..23: mol_type = other RNA
actggagacacgtgcactgtaga

SEQ ID NO: 46 - RNA, 23 nt, Homo sapiens
  source 1..23: mol_type = other RNA
gggagtgaagacacggagccaga

SEQ ID NO: 47 - RNA, 22 nt, Homo sapiens
  source 1..22: mol_type = other RNA
gatcacttttgtgactatgcaa

SEQ ID NO: 48 - RNA, 22 nt, Homo sapiens
  source 1..22: mol_type = other RNA
agtgaattctaccagtgccata

SEQ ID NO: 49 - RNA, 22 nt, Homo sapiens
  source 1..22: mol_type = other RNA
acctaatatatcaaacatatca

SEQ ID NO: 50 - RNA, 21 nt, Homo sapiens
  source 1..21: mol_type = other RNA
agaattgcgtttggacaatca

SEQ ID NO: 51 - RNA, 22 nt, Homo sapiens
  source 1..22: mol_type = other RNA
cgccaatatttacgtgctgcta

SEQ ID NO: 52 - RNA, 22 nt, Homo sapiens
  source 1..22: mol_type = other RNA
tcaacatcagtctgataagcta

SEQ ID NO: 53 - RNA, 22 nt, Homo sapiens
  source 1..22: mol_type = other RNA
ctgttcctgctgaactgagcca

SEQ ID NO: 54 - RNA, 21 nt, Homo sapiens
  source 1..21: mol_type = other RNA
gcggaacttagccactgtgaa

SEQ ID NO: 55 - RNA, 22 nt, Homo sapiens
  source 1..22: mol_type = other RNA
cacaagatcggatctacgggtt

SEQ ID NO: 56 - RNA, 22 nt, Homo sapiens
  source 1..22: mol_type = other RNA
agccaagctcagacggatccga

SEQ ID NO: 57 - RNA, 22 nt, Homo sapiens
  source 1..22: mol_type = other RNA
cgaccatggctgtagactgtta

SEQ ID NO: 58 - RNA, 23 nt, Homo sapiens
  source 1..23: mol_type = other RNA
tccataaagtaggaaacactaca

SEQ ID NO: 59 - RNA, 21 nt, Homo sapiens
  source 1..21: mol_type = other RNA
actagactgtgagctcctcga

SEQ ID NO: 60 - RNA, 23 nt, Homo sapiens
  source 1..23: mol_type = other RNA
actcaccgacagcgttgaatgtt

SEQ ID NO: 61 - RNA, 22 nt, Homo sapiens
  source 1..22: mol_type = other RNA
actgatatcagctcagtaggca

SEQ ID NO: 62 - RNA, 23 nt, Homo sapiens
  source 1..23: mol_type = other RNA
agtaagcagtctagagccaaggt

SEQ ID NO: 63 - RNA, 22 nt, Homo sapiens
  source 1..22: mol_type = other RNA
tggggtatttgacaaactgaca

SEQ ID NO: 64 - RNA, 23 nt, Homo sapiens
  source 1..23: mol_type = other RNA
ctacctgcactgtaagcactttg

SEQ ID NO: 65 - RNA, 22 nt, Homo sapiens
  source 1..22: mol_type = other RNA
acaggccgggacaagtgcaata

SEQ ID NO: 66 - RNA, 21 nt, Homo sapiens
  source 1..21: mol_type = other RNA
cgcgtaccaaaagtaataatg

SEQ ID NO: 67 - RNA, 141 nt, synthetic construct
  misc_feature 1..141: note = sequence of expression regulatory element
  source 1..141: mol_type = other RNA
tgataataggctggagcctcggtggccatgcttcttgccccttgggcctccccccagcccctcctccccttcctgcacccgtaccccccaaacaccattgtcacactccagtggtctttgaataaagtctgagtgggcggc

SEQ ID NO: 68 - RNA, 185 nt, synthetic construct
  misc_feature 1..185: note = sequence of expression regulatory element
  source 1..185: mol_type = other RNA
tgataatagcaaacaccattgtcacactccagctggagcctcggtggccatgcttcttgccccttgggcccaaacaccattgtcacactccatccccccagcccctcctccccttcctgcacccgtaccccccaaacaccattgtcacactccagtggtctttgaataaagtctgagtgggcggc

SEQ ID NO: 69 - RNA, 2691 nt, synthetic construct
  misc_feature 1..2691: note = sequence of circular RNA molecule
  source 1..2691: mol_type = other RNA
aaaatccgttgaccttaaacggtcgtgtgggttcaagtccctccacccccacgccggaaacgcaatagccgaaaaaacaaaaacaaaaaaaacaaaaaaacaaaaaaaaaaccaaaacacattaaaacagcctgtgggttgatcccacccacagggcccactgggcgctagcactctggtatcacggtacctttgtgcgcctgttttatacttcctcccccaactgcaacttagaagtaacacaaaccgatcaacagtcagcgtggcacaccagccacgttttgatcaaacacttctgttaccccggactgagtatcaatagactgctcacgcggttgaaggagaaaacgttcgttatccggccaactacttcgagaaacctagtaacgccatggaagttgtggagtgtttcgctcagcactaccccagtgtagatcaggttgatgagtcaccgcattccccacgggtgaccgtggcggtggctgcgttggcggcctgcccatggggaaacccatgggacgctcttatacagacatggtgcgaagagtctattgagctagttggtagtcctccggcccctgaatgcggctaatcccaactgcggagcatacactctcaagccagagggtagtgtgtcgtaatgggcaactctgcagcggaaccgactactttgggtgtccgtgtttcattttattcctatactggctgcttatggtgacaattgagagattgttaccatatagctattggattggccatccggtgactaacagagctattatatatctttttgttgggtttataccacttagcttgaaagaggttaaaactctacattacattttaatactgaacaccgcaaaatggaggacgccaagaacatcaagaagggccctgcccctttctaccctctggaggacggcaccgccggcgagcagctgcacaaggccatgaagaggtacgccctggtgcctggcaccatcgccttcaccgacgcccacatcgaggtggacatcacctacgccgagtacttcgagatgagcgtgaggctggccgaggccatgaagaggtacggcctgaacaccaaccacaggatcgtggtgtgcagcgagaacagcctgcagttcttcatgcctgtgctgggcgccctgttcatcggcgtggccgtggcccctgccaacgacatctacaacgagagggagctgctgaacagcatgggcatcagccagcctaccgtggtgttcgtgagcaagaagggcctgcagaagatcctgaacgtgcagaagaagctgcctatcatccagaagatcatcatcatggacagcaagaccgactaccagggcttccagagcatgtacaccttcgtgaccagccacctgcctcctggcttcaacgagtacgacttcgtgcctgagagcttcgacagggacaagaccatcgccctgatcatgaacagcagcggcagcaccggcctgcctaagggcgtggccctgcctcacaggaccgcctgcgtgaggttcagccacgccagggaccctatcttcggcaaccagatcatccctgacaccgccatcctgagcgtggtgcctttccaccacggcttcggcatgttcaccaccctgggctacctgatctgcggcttcagggtggtgctgatgtacaggttcgaggaggagctgttcctgaggagcctgcaggactacaagatccagagcgccctgctggtgcctaccctgttcagcttcttcgccaagagcaccctgatcgacaagtacgacctgagcaacctgcacgagatcgccagcggcggcgcccctctgagcaaggaggtgggcgaggccgtggccaagaggttccacctgcctggcatcaggcagggctacggcctgaccgagaccaccagcgccatcctgatcacccctgagggcgacgacaagcctggcgccgtgggcaaggtggtgcctttcttcgaggccaaggtggtggacctggacaccggcaagaccctgggcgtgaaccagaggggcgagctgtgcgtgaggggccctatgatcatgagcggctacgtgaacaaccctgaggccaccaacgccctgatcgacaaggacggctggctgcacagcggcgacatcgcctactgggacgaggacgagcacttcttcatcgtggacaggctgaagagcctgatcaagtacaagggctaccaggtggcccctgccgagctggagagcatcctgctgcagcaccctaacatcttcgacgccggcgtggctggcttgcctgatgacgatgctggagagctgcctgccgccgtggtggtgctggagcacggcaagaccatgaccgagaaggagatcgtggactacgtggccagccaggtgaccaccgccaagaagctgaggggcggcgtggtgttcgtggacgaggtgcctaagggcctgaccggcaagctggacgccaggaagatcagggagatcctgatcaaggccaagaagggcggcaagatcgccgtgtgatgataataggctggagcctcggtggccatgcttcttgccccttgggcctccccccagcccctcctccccttcctgcacccgtacccccgtggtctttgaataaagtctgagtgggcggcaaaaaacaaaaaacaaaacggctattatgcgttaccggcgagacgctacggactta

SEQ ID NO: 70 - RNA, 2713 nt, synthetic construct
  misc_feature 1..2713: note = sequence of circular RNA molecule
  source 1..2713: mol_type = other RNA
aaaatccgttgaccttaaacggtcgtgtgggttcaagtccctccacccccacgccggaaacgcaatagccgaaaaaacaaaaacaaaaaaaacaaaaaaacaaaaaaaaaaccaaaacacattaaaacagcctgtgggttgatcccacccacagggcccactgggcgctagcactctggtatcacggtacctttgtgcgcctgttttatacttcctcccccaactgcaacttagaagtaacacaaaccgatcaacagtcagcgtggcacaccagccacgttttgatcaaacacttctgttaccccggactgagtatcaatagactgctcacgcggttgaaggagaaaacgttcgttatccggccaactacttcgagaaacctagtaacgccatggaagttgtggagtgtttcgctcagcactaccccagtgtagatcaggttgatgagtcaccgcattccccacgggtgaccgtggcggtggctgcgttggcggcctgcccatggggaaacccatgggacgctcttatacagacatggtgcgaagagtctattgagctagttggtagtcctccggcccctgaatgcggctaatcccaactgcggagcatacactctcaagccagagggtagtgtgtcgtaatgggcaactctgcagcggaaccgactactttgggtgtccgtgtttcattttattcctatactggctgcttatggtgacaattgagagattgttaccatatagctattggattggccatccggtgactaacagagctattatatatctttttgttgggtttataccacttagcttgaaagaggttaaaactctacattacattttaatactgaacaccgcaaaatggaggacgccaagaacatcaagaagggccctgcccctttctaccctctggaggacggcaccgccggcgagcagctgcacaaggccatgaagaggtacgccctggtgcctggcaccatcgccttcaccgacgcccacatcgaggtggacatcacctacgccgagtacttcgagatgagcgtgaggctggccgaggccatgaagaggtacggcctgaacaccaaccacaggatcgtggtgtgcagcgagaacagcctgcagttcttcatgcctgtgctgggcgccctgttcatcggcgtggccgtggcccctgccaacgacatctacaacgagagggagctgctgaacagcatgggcatcagccagcctaccgtggtgttcgtgagcaagaagggcctgcagaagatcctgaacgtgcagaagaagctgcctatcatccagaagatcatcatcatggacagcaagaccgactaccagggcttccagagcatgtacaccttcgtgaccagccacctgcctcctggcttcaacgagtacgacttcgtgcctgagagcttcgacagggacaagaccatcgccctgatcatgaacagcagcggcagcaccggcctgcctaagggcgtggccctgcctcacaggaccgcctgcgtgaggttcagccacgccagggaccctatcttcggcaaccagatcatccctgacaccgccatcctgagcgtggtgcctttccaccacggcttcggcatgttcaccaccctgggctacctgatctgcggcttcagggtggtgctgatgtacaggttcgaggaggagctgttcctgaggagcctgcaggactacaagatccagagcgccctgctggtgcctaccctgttcagcttcttcgccaagagcaccctgatcgacaagtacgacctgagcaacctgcacgagatcgccagcggcggcgcccctctgagcaaggaggtgggcgaggccgtggccaagaggttccacctgcctggcatcaggcagggctacggcctgaccgagaccaccagcgccatcctgatcacccctgagggcgacgacaagcctggcgccgtgggcaaggtggtgcctttcttcgaggccaaggtggtggacctggacaccggcaagaccctgggcgtgaaccagaggggcgagctgtgcgtgaggggccctatgatcatgagcggctacgtgaacaaccctgaggccaccaacgccctgatcgacaaggacggctggctgcacagcggcgacatcgcctactgggacgaggacgagcacttcttcatcgtggacaggctgaagagcctgatcaagtacaagggctaccaggtggcccctgccgagctggagagcatcctgctgcagcaccctaacatcttcgacgccggcgtggctggcttgcctgatgacgatgctggagagctgcctgccgccgtggtggtgctggagcacggcaagaccatgaccgagaaggagatcgtggactacgtggccagccaggtgaccaccgccaagaagctgaggggcggcgtggtgttcgtggacgaggtgcctaagggcctgaccggcaagctggacgccaggaagatcagggagatcctgatcaaggccaagaagggcggcaagatcgccgtgtgatgataataggctggagcctcggtggccatgcttcttgccccttgggcctccccccagcccctcctccccttcctgcacccgtaccccccaaacaccattgtcacactccagtggtctttgaataaagtctgagtgggcggcaaaaaacaaaaaacaaaacggctattatgcgttaccggcgagacgctacggactta

SEQ ID NO: 71 - RNA, 2757 nt, synthetic construct
  misc_feature 1..2757: note = sequence of circular RNA molecule
  source 1..2757: mol_type = other RNA
aaaatccgttgaccttaaacggtcgtgtgggttcaagtccctccacccccacgccggaaacgcaatagccgaaaaaacaaaaacaaaaaaaacaaaaaaacaaaaaaaaaaccaaaacacattaaaacagcctgtgggttgatcccacccacagggcccactgggcgctagcactctggtatcacggtacctttgtgcgcctgttttatacttcctcccccaactgcaacttagaagtaacacaaaccgatcaacagtcagcgtggcacaccagccacgttttgatcaaacacttctgttaccccggactgagtatcaatagactgctcacgcggttgaaggagaaaacgttcgttatccggccaactacttcgagaaacctagtaacgccatggaagttgtggagtgtttcgctcagcactaccccagtgtagatcaggttgatgagtcaccgcattccccacgggtgaccgtggcggtggctgcgttggcggcctgcccatggggaaacccatgggacgctcttatacagacatggtgcgaagagtctattgagctagttggtagtcctccggcccctgaatgcggctaatcccaactgcggagcatacactctcaagccagagggtagtgtgtcgtaatgggcaactctgcagcggaaccgactactttgggtgtccgtgtttcattttattcctatactggctgcttatggtgacaattgagagattgttaccatatagctattggattggccatccggtgactaacagagctattatatatctttttgttgggtttataccacttagcttgaaagaggttaaaactctacattacattttaatactgaacaccgcaaaatggaggacgccaagaacatcaagaagggccctgcccctttctaccctctggaggacggcaccgccggcgagcagctgcacaaggccatgaagaggtacgccctggtgcctggcaccatcgccttcaccgacgcccacatcgaggtggacatcacctacgccgagtacttcgagatgagcgtgaggctggccgaggccatgaagaggtacggcctgaacaccaaccacaggatcgtggtgtgcagcgagaacagcctgcagttcttcatgcctgtgctgggcgccctgttcatcggcgtggccgtggcccctgccaacgacatctacaacgagagggagctgctgaacagcatgggcatcagccagcctaccgtggtgttcgtgagcaagaagggcctgcagaagatcctgaacgtgcagaagaagctgcctatcatccagaagatcatcatcatggacagcaagaccgactaccagggcttccagagcatgtacaccttcgtgaccagccacctgcctcctggcttcaacgagtacgacttcgtgcctgagagcttcgacagggacaagaccatcgccctgatcatgaacagcagcggcagcaccggcctgcctaagggcgtggccctgcctcacaggaccgcctgcgtgaggttcagccacgccagggaccctatcttcggcaaccagatcatccctgacaccgccatcctgagcgtggtgcctttccaccacggcttcggcatgttcaccaccctgggctacctgatctgcggcttcagggtggtgctgatgtacaggttcgaggaggagctgttcctgaggagcctgcaggactacaagatccagagcgccctgctggtgcctaccctgttcagcttcttcgccaagagcaccctgatcgacaagtacgacctgagcaacctgcacgagatcgccagcggcggcgcccctctgagcaaggaggtgggcgaggccgtggccaagaggttccacctgcctggcatcaggcagggctacggcctgaccgagaccaccagcgccatcctgatcacccctgagggcgacgacaagcctggcgccgtgggcaaggtggtgcctttcttcgaggccaaggtggtggacctggacaccggcaagaccctgggcgtgaaccagaggggcgagctgtgcgtgaggggccctatgatcatgagcggctacgtgaacaaccctgaggccaccaacgccctgatcgacaaggacggctggctgcacagcggcgacatcgcctactgggacgaggacgagcacttcttcatcgtggacaggctgaagagcctgatcaagtacaagggctaccaggtggcccctgccgagctggagagcatcctgctgcagcaccctaacatcttcgacgccggcgtggctggcttgcctgatgacgatgctggagagctgcctgccgccgtggtggtgctggagcacggcaagaccatgaccgagaaggagatcgtggactacgtggccagccaggtgaccaccgccaagaagctgaggggcggcgtggtgttcgtggacgaggtgcctaagggcctgaccggcaagctggacgccaggaagatcagggagatcctgatcaaggccaagaagggcggcaagatcgccgtgtgatgataatagcaaacaccattgtcacactccagctggagcctcggtggccatgcttcttgccccttgggcccaaacaccattgtcacactccatccccccagcccctcctccccttcctgcacccgtaccccccaaacaccattgtcacactccagtggtctttgaataaagtctgagtgggcggcaaaaaacaaaaaacaaaacggctattatgcgttaccggcgagacgctacggactta

SEQ ID NO: 72 - RNA, 1545 nt, synthetic construct
  misc_feature 1..1545: note = sequence of circular RNA molecule
  source 1..1545: mol_type = other RNA
aaaatccgttgaccttaaacggtcgtgtgggttcaagtccctccacccccacgccggaaacgcaatagccgaaaaaacaaaaacaaaaaaaacaaaaaaacaaaaaaaaaaccaaaacacattaaaacagcctgtgggttgatcccacccacagggcccactgggcgctagcactctggtatcacggtacctttgtgcgcctgttttatacttcctcccccaactgcaacttagaagtaacacaaaccgatcaacagtcagcgtggcacaccagccacgttttgatcaaacacttctgttaccccggactgagtatcaatagactgctcacgcggttgaaggagaaaacgttcgttatccggccaactacttcgagaaacctagtaacgccatggaagttgtggagtgtttcgctcagcactaccccagtgtagatcaggttgatgagtcaccgcattccccacgggtgaccgtggcggtggctgcgttggcggcctgcccatggggaaacccatgggacgctcttatacagacatggtgcgaagagtctattgagctagttggtagtcctccggcccctgaatgcggctaatcccaactgcggagcatacactctcaagccagagggtagtgtgtcgtaatgggcaactctgcagcggaaccgactactttgggtgtccgtgtttcattttattcctatactggctgcttatggtgacaattgagagattgttaccatatagctattggattggccatccggtgactaacagagctattatatatctttttgttgggtttataccacttagcttgaaagaggttaaaactctacattacattttaatactgaacaccgcaaaatgtacagcatgcagctggccagctgcgtgaccctgaccctggtgctgctggtgaacagcgcccccaccagcagcagcaccagcagcagcaccgccgaggcccagcagcagcagcagcagcagcagcagcagcagcagcacctggagcagctgctgatggacctgcaggagctgctgagcaggatggagaactacaggaacctgaagctgcccaggatgctgaccttcaagttctacctgcccaagcaggccaccgagctgaaggacctgcagtgcctggaggacgagctgggccccctgaggcacgtgctggacctgacccagagcaagagcttccagctggaggacgccgagaacttcatcagcaacatcagggtgaccgtggtgaagctgaagggcagcgacaacaccttcgagtgccagttcgacgacgagagcgccaccgtggtggacttcctgaggaggtggatcgccttctgccagagcatcatcagcaccagcccccagtgataataggctggagcctcggtggccatgcttcttgccccttgggcctccccccagcccctcctccccttcctgcacccgtacccccgtggtctttgaataaagtctgagtgggcggcaaaaaacaaaaaacaaaacggctattatgcgttaccggcgagacgctacggactta

SEQ ID NO: 73 - RNA, 1611 nt, synthetic construct
  misc_feature 1..1611: note = sequence of circular RNA molecule
  source 1..1611: mol_type = other RNA
aaaatccgttgaccttaaacggtcgtgtgggttcaagtccctccacccccacgccggaaacgcaatagccgaaaaaacaaaaacaaaaaaaacaaaaaaacaaaaaaaaaaccaaaacacattaaaacagcctgtgggttgatcccacccacagggcccactgggcgctagcactctggtatcacggtacctttgtgcgcctgttttatacttcctcccccaactgcaacttagaagtaacacaaaccgatcaacagtcagcgtggcacaccagccacgttttgatcaaacacttctgttaccccggactgagtatcaatagactgctcacgcggttgaaggagaaaacgttcgttatccggccaactacttcgagaaacctagtaacgccatggaagttgtggagtgtttcgctcagcactaccccagtgtagatcaggttgatgagtcaccgcattccccacgggtgaccgtggcggtggctgcgttggcggcctgcccatggggaaacccatgggacgctcttatacagacatggtgcgaagagtctattgagctagttggtagtcctccggcccctgaatgcggctaatcccaactgcggagcatacactctcaagccagagggtagtgtgtcgtaatgggcaactctgcagcggaaccgactactttgggtgtccgtgtttcattttattcctatactggctgcttatggtgacaattgagagattgttaccatatagctattggattggccatccggtgactaacagagctattatatatctttttgttgggtttataccacttagcttgaaagaggttaaaactctacattacattttaatactgaacaccgcaaaatgtacagcatgcagctggccagctgcgtgaccctgaccctggtgctgctggtgaacagcgcccccaccagcagcagcaccagcagcagcaccgccgaggcccagcagcagcagcagcagcagcagcagcagcagcagcacctggagcagctgctgatggacctgcaggagctgctgagcaggatggagaactacaggaacctgaagctgcccaggatgctgaccttcaagttctacctgcccaagcaggccaccgagctgaaggacctgcagtgcctggaggacgagctgggccccctgaggcacgtgctggacctgacccagagcaagagcttccagctggaggacgccgagaacttcatcagcaacatcagggtgaccgtggtgaagctgaagggcagcgacaacaccttcgagtgccagttcgacgacgagagcgccaccgtggtggacttcctgaggaggtggatcgccttctgccagagcatcatcagcaccagcccccagtgataatagcaaacaccattgtcacactccagctggagcctcggtggccatgcttcttgccccttgggcccaaacaccattgtcacactccatccccccagcccctcctccccttcctgcacccgtaccccccaaacaccattgtcacactccagtggtctttgaataaagtctgagtgggcggcaaaaaacaaaaaacaaaacggctattatgcgttaccggcgagacgctacggactta

SEQ ID NO: 74 - RNA, 2382 nt, synthetic construct
  misc_feature 1..2382: note = sequence of circular RNA molecule
  source 1..2382: mol_type = other RNA
aaaatccgttgaccttaaacggtcgtgtgggttcaagtccctccacccccacgccggaaacgcaatagccgaaaaaacaaaaacaaaaaaaacaaaaaaacaaaaaaaaaaccaaaacacattaaaacagcctgtgggttgatcccacccacagggcccactgggcgctagcactctggtatcacggtacctttgtgcgcctgttttatacttcctcccccaactgcaacttagaagtaacacaaaccgatcaacagtcagcgtggcacaccagccacgttttgatcaaacacttctgttaccccggactgagtatcaatagactgctcacgcggttgaaggagaaaacgttcgttatccggccaactacttcgagaaacctagtaacgccatggaagttgtggagtgtttcgctcagcactaccccagtgtagatcaggttgatgagtcaccgcattccccacgggtgaccgtggcggtggctgcgttggcggcctgcccatggggaaacccatgggacgctcttatacagacatggtgcgaagagtctattgagctagttggtagtcctccggcccctgaatgcggctaatcccaactgcggagcatacactctcaagccagagggtagtgtgtcgtaatgggcaactctgcagcggaaccgactactttgggtgtccgtgtttcattttattcctatactggctgcttatggtgacaattgagagattgttaccatatagctattggattggccatccggtgactaacagagctattatatatctttttgttgggtttataccacttagcttgaaagaggttaaaactctacattacattttaatactgaacaccgcaaacaggtgcagctggtggagagcggcggcggcgtggtgcagcccggcaggagcctgaggctgagctgcgccgccagcggcttcaccttcagcagctacaccatgcactgggtgaggcaggcccccggcaagggcctggagtgggtgaccttcatcagctacgacggcaacaacaagtactacgccgacagcgtgaagggcaggttcaccatcagcagggacaacagcaagaacaccctgtacctgcagatgaacagcctgagggccgaggacaccgccatctactactgcgccaggaccggctggctgggccccttcgactactggggccagggcaccctggtgaccgtgagcagcgccagcaccaagggccccagcgtgttccccctggcccccagcagcaagagcaccagcggcggcaccgccgccctgggctgcctggtgaaggactacttccccgagcccgtgaccgtgagctggaacagcggcgccctgaccagcggcgtgcacaccttccccgccgtgctgcagagcagcggcctgtacagcctgagcagcgtggtgaccgtgcccagcagcagcctgggcacccagacctacatctgcaacgtgaaccacaagcccagcaacaccaaggtggacaagagggtggagcccaagagctgcgacaagacccacacctgccccccctgccccgcccccgagctgctgggcggccccagcgtgttcctgttcccccccaagcccaaggacaccctgatgatcagcaggacccccgaggtgacctgcgtggtggtggacgtgagccacgaggaccccgaggtgaagttcaactggtacgtggacggcgtggaggtgcacaacgccaagaccaagcccagggaggagcagtacaacagcacctacagggtggtgagcgtgctgaccgtgctgcaccaggactggctgaacggcaaggagtacaagtgcaaggtgagcaacaaggccctgcccgcccccatcgagaagaccatcagcaaggccaagggccagcccagggagccccaggtgtacaccctgccccccagcagggacgagctgaccaagaaccaggtgagcctgacctgcctggtgaagggcttctaccccagcgacatcgccgtggagtgggagagcaacggccagcccgagaacaactacaagaccaccccccccgtgctggacagcgacggcagcttcttcctgtacagcaagctgaccgtggacaagagcaggtggcagcagggcaacgtgttcagctgcagcgtgatgcacgaggccctgcacaaccactacacccagaagagcctgagcctgagccccggcaagtgataataggctggagcctcggtggccatgcttcttgccccttgggcctccccccagcccctcctccccttcctgcacccgtacccccgtggtctttgaataaagtctgagtgggcggcaaaaaacaaaaaacaaaacggctattatgcgttaccggcgagacgctacggactta

SEQ ID NO: 75 - RNA, 1683 nt, synthetic construct
  misc_feature 1..1683: note = sequence of circular RNA molecule
  source 1..1683: mol_type = other RNA
aaaatccgttgaccttaaacggtcgtgtgggttcaagtccctccacccccacgccggaaacgcaatagccgaaaaaacaaaaacaaaaaaaacaaaaaaacaaaaaaaaaaccaaaacacattaaaacagcctgtgggttgatcccacccacagggcccactgggcgctagcactctggtatcacggtacctttgtgcgcctgttttatacttcctcccccaactgcaacttagaagtaacacaaaccgatcaacagtcagcgtggcacaccagccacgttttgatcaaacacttctgttaccccggactgagtatcaatagactgctcacgcggttgaaggagaaaacgttcgttatccggccaactacttcgagaaacctagtaacgccatggaagttgtggagtgtttcgctcagcactaccccagtgtagatcaggttgatgagtcaccgcattccccacgggtgaccgtggcggtggctgcgttggcggcctgcccatggggaaacccatgggacgctcttatacagacatggtgcgaagagtctattgagctagttggtagtcctccggcccctgaatgcggctaatcccaactgcggagcatacactctcaagccagagggtagtgtgtcgtaatgggcaactctgcagcggaaccgactactttgggtgtccgtgtttcattttattcctatactggctgcttatggtgacaattgagagattgttaccatatagctattggattggccatccggtgactaacagagctattatatatctttttgttgggtttataccacttagcttgaaagaggttaaaactctacattacattttaatactgaacaccgcaaagagatcgtgctgacccagagccccggcaccctgagcctgagccccggcgagagggccaccctgagctgcagggccagccagagcgtgggcagcagctacctggcctggtaccagcagaagcccggccaggcccccaggctgctgatctacggcgccttcagcagggccaccggcatccccgacaggttcagcggcagcggcagcggcaccgacttcaccctgaccatcagcaggctggagcccgaggacttcgccgtgtactactgccagcagtacggcagcagcccctggaccttcggccagggcaccaaggtggagatcaagaggaccgtggccgcccccagcgtgttcatcttcccccccagcgacgagcagctgaagagcggcaccgccagcgtggtgtgcctgctgaacaacttctaccccagggaggccaaggtgcagtggaaggtggacaacgccctgcagagcggcaacagccaggagagcgtgaccgagcaggacagcaaggacagcacctacagcctgagcagcaccctgaccctgagcaaggccgactacgagaagcacaaggtgtacgcctgcgaggtgacccaccagggcctgagcagccccgtgaccaagagcttcaacaggggcgagtgctgataataggctggagcctcggtggccatgcttcttgccccttgggcctccccccagcccctcctccccttcctgcacccgtacccccgtggtctttgaataaagtctgagtgggcggcaaaaaacaaaaaacaaaacggctattatgcgttaccggcgagacgctacggactta

SEQ ID NO: 76 - RNA, 2448 nt, synthetic construct
  misc_feature 1..2448: note = sequence of circular RNA molecule
  source 1..2448: mol_type = other RNA
aaaatccgttgaccttaaacggtcgtgtgggttcaagtccctccacccccacgccggaaacgcaatagccgaaaaaacaaaaacaaaaaaaacaaaaaaacaaaaaaaaaaccaaaacacattaaaacagcctgtgggttgatcccacccacagggcccactgggcgctagcactctggtatcacggtacctttgtgcgcctgttttatacttcctcccccaactgcaacttagaagtaacacaaaccgatcaacagtcagcgtggcacaccagccacgttttgatcaaacacttctgttaccccggactgagtatcaatagactgctcacgcggttgaaggagaaaacgttcgttatccggccaactacttcgagaaacctagtaacgccatggaagttgtggagtgtttcgctcagcactaccccagtgtagatcaggttgatgagtcaccgcattccccacgggtgaccgtggcggtggctgcgttggcggcctgcccatggggaaacccatgggacgctcttatacagacatggtgcgaagagtctattgagctagttggtagtcctccggcccctgaatgcggctaatcccaactgcggagcatacactctcaagccagagggtagtgtgtcgtaatgggcaactctgcagcggaaccgactactttgggtgtccgtgtttcattttattcctatactggctgcttatggtgacaattgagagattgttaccatatagctattggattggccatccggtgactaacagagctattatatatctttttgttgggtttataccacttagcttgaaagaggttaaaactctacattacattttaatactgaacaccgcaaacaggtgcagctggtggagagcggcggcggcgtggtgcagcccggcaggagcctgaggctgagctgcgccgccagcggcttcaccttcagcagctacaccatgcactgggtgaggcaggcccccggcaagggcctggagtgggtgaccttcatcagctacgacggcaacaacaagtactacgccgacagcgtgaagggcaggttcaccatcagcagggacaacagcaagaacaccctgtacctgcagatgaacagcctgagggccgaggacaccgccatctactactgcgccaggaccggctggctgggccccttcgactactggggccagggcaccctggtgaccgtgagcagcgccagcaccaagggccccagcgtgttccccctggcccccagcagcaagagcaccagcggcggcaccgccgccctgggctgcctggtgaaggactacttccccgagcccgtgaccgtgagctggaacagcggcgccctgaccagcggcgtgcacaccttccccgccgtgctgcagagcagcggcctgtacagcctgagcagcgtggtgaccgtgcccagcagcagcctgggcacccagacctacatctgcaacgtgaaccacaagcccagcaacaccaaggtggacaagagggtggagcccaagagctgcgacaagacccacacctgccccccctgccccgcccccgagctgctgggcggccccagcgtgttcctgttcccccccaagcccaaggacaccctgatgatcagcaggacccccgaggtgacctgcgtggtggtggacgtgagccacgaggaccccgaggtgaagttcaactggtacgtggacggcgtggaggtgcacaacgccaagaccaagcccagggaggagcagtacaacagcacctacagggtggtgagcgtgctgaccgtgctgcaccaggactggctgaacggcaaggagtacaagtgcaaggtgagcaacaaggccctgcccgcccccatcgagaagaccatcagcaaggccaagggccagcccagggagccccaggtgtacaccctgccccccagcagggacgagctgaccaagaaccaggtgagcctgacctgcctggtgaagggcttctaccccagcgacatcgccgtggagtgggagagcaacggccagcccgagaacaactacaagaccaccccccccgtgctggacagcgacggcagcttcttcctgtacagcaagctgaccgtggacaagagcaggtggcagcagggcaacgtgttcagctgcagcgtgatgcacgaggccctgcacaaccactacacccagaagagcctgagcctgagccccggcaagtgataatagcaaacaccattgtcacactccagctggagcctcggtggccatgcttcttgccccttgggcccaaacaccattgtcacactccatccccccagcccctcctccccttcctgcacccgtaccccccaaacaccattgtcacactccagtggtctttgaataaagtctgagtgggcggcaaaaaacaaaaaacaaaacggctattatgcgttaccggcgagacgctacggactta

SEQ ID NO: 77 - RNA, 1749 nt, synthetic construct
  misc_feature 1..1749: note = sequence of circular RNA molecule
  source 1..1749: mol_type = other RNA
aaaatccgttgaccttaaacggtcgtgtgggttcaagtccctccacccccacgccggaaacgcaatagccgaaaaaacaaaaacaaaaaaaacaaaaaaacaaaaaaaaaaccaaaacacattaaaacagcctgtgggttgatcccacccacagggcccactgggcgctagcactctggtatcacggtacctttgtgcgcctgttttatacttcctcccccaactgcaacttagaagtaacacaaaccgatcaacagtcagcgtggcacaccagccacgttttgatcaaacacttctgttaccccggactgagtatcaatagactgctcacgcggttgaaggagaaaacgttcgttatccggccaactacttcgagaaacctagtaacgccatggaagttgtggagtgtttcgctcagcactaccccagtgtagatcaggttgatgagtcaccgcattccccacgggtgaccgtggcggtggctgcgttggcggcctgcccatggggaaacccatgggacgctcttatacagacatggtgcgaagagtctattgagctagttggtagtcctccggcccctgaatgcggctaatcccaactgcggagcatacactctcaagccagagggtagtgtgtcgtaatgggcaactctgcagcggaaccgactactttgggtgtccgtgtttcattttattcctatactggctgcttatggtgacaattgagagattgttaccatatagctattggattggccatccggtgactaacagagctattatatatctttttgttgggtttataccacttagcttgaaagaggttaaaactctacattacattttaatactgaacaccgcaaagagatcgtgctgacccagagccccggcaccctgagcctgagccccggcgagagggccaccctgagctgcagggccagccagagcgtgggcagcagctacctggcctggtaccagcagaagcccggccaggcccccaggctgctgatctacggcgccttcagcagggccaccggcatccccgacaggttcagcggcagcggcagcggcaccgacttcaccctgaccatcagcaggctggagcccgaggacttcgccgtgtactactgccagcagtacggcagcagcccctggaccttcggccagggcaccaaggtggagatcaagaggaccgtggccgcccccagcgtgttcatcttcccccccagcgacgagcagctgaagagcggcaccgccagcgtggtgtgcctgctgaacaacttctaccccagggaggccaaggtgcagtggaaggtggacaacgccctgcagagcggcaacagccaggagagcgtgaccgagcaggacagcaaggacagcacctacagcctgagcagcaccctgaccctgagcaaggccgactacgagaagcacaaggtgtacgcctgcgaggtgacccaccagggcctgagcagccccgtgaccaagagcttcaacaggggcgagtgctgataatagcaaacaccattgtcacactccagctggagcctcggtggccatgcttcttgccccttgggcccaaacaccattgtcacactccatccccccagcccctcctccccttcctgcacccgtaccccccaaacaccattgtcacactccagtggtctttgaataaagtctgagtgggcggcaaaaaacaaaaaacaaaacggctattatgcgttaccggcgagacgctacggactta

SEQ ID NO: 78 - RNA, 741 nt, synthetic construct
  misc_feature 1..741: note = sequence of IRES element
  source 1..741: mol_type = other RNA
ttaaaacagcctgtgggttgatcccacccacaggcccattgggcgctagcactctggtatcacggtacctttgtgcgcctgttttataccccctcccccaactgtaacttagaagtaacacacaccgatcaacagtcagcgtggcacaccagccacgttttgatcaagcacttctgttaccccggactgagtatcaatagactgctcacgcggttgaaggagaaagcgttcgttatccggccaactacttcgaaaaacctagtaacaccgtggaagttgcagagtgtttcgctcagcactaccccagtgtagatcaggtcgatgagtcaccgcattccccacgggcgaccgtggcggtggctgcgttggcggcctgcccatggggaaacccatgggacgctctaatacagacatggtgcgaagagtctattgagctagttggtagtcctccggcccctgaatgcggctaatcctaactgcggagcacacaccctcaagccagagggcagtgtgtcgtaacgggcaactctgcagcggaaccgactactttgggtgtccgtgtttcattttattcctatactggctgcttatggtgacaattgagagatcgttaccatatagctattggattggccatccggtgactaatagagctattatatatccctttgttgggtttataccacttagcttgaaagaggttaaaacattacaattcattgttaagttgaatacagcaaa

SEQ ID NO: 79 - RNA, 682 nt, synthetic construct
  misc_feature 1..682: note = sequence of IRES element
  source 1..682: mol_type = other RNA
ttaaaacagcctgtgggttgcacccacccacagggcccacagggcgctagcactctggtatcacggtacctttgtgcgcctgttttattaccccttccccaattgaaaattagaagcaatgcacaccgatcaacagcaggcgtggcgcaccagtcacgtctcgatcaagcacttctgtttccccggaccgagtatcaatagactgctcacgcggttgaaggagaaagtgttcgttatccggctaaccacttcgagaaacccagtaacaccatgaaagttgcagggtgtttcgctcagcacttccccagtgtagatcaggtcgatgagtcaccgcgttccccacgggcgaccgtggcggtggctgcgttggcggcctgcctatgggttaacccataggacgctctaatacagacatggtgcgaagagtttattgagctggttagtatccctccggcccctgaatgcggctaatcctaactgcggagcacgtgcctccaatccagggggttgcatgtcgtaacgggtaactctgcagcggaaccgactactttgggtgtccgtgtttccttttattcttatactggctgcttatggtgacaatcgaggaattgttaccatatagctattggattggccatccggtgtctaacagagcgattatatacctctttgttggatttat

SEQ ID NO: 80 - RNA, 742 nt, synthetic construct
  misc_feature 1..742: note = sequence of IRES element
  source 1..742: mol_type = other RNA
ttaaaacagcctgtgggttgatcccacccacagggcccactgggcgctagcactctggtatcacggtacctttgtgcgcctgttttatacttcctcccccaactgcaacttagaagtaacacaaaccgatcaacagtcagcgtggcacaccagccacgttttgatcaaacacttctgttaccccggactgagtatcaatagactgctcacgcggttgaaggagaaaacgttcgttatccggccaactacttcgagaaacctagtaacgccatggaagttgtggagtgtttcgctcagcactaccccagtgtagatcaggttgatgagtcaccgcattccccacgggtgaccgtggcggtggctgcgttggcggcctgcccatggggaaacccatgggacgctcttatacagacatggtgcgaagagtctattgagctagttggtagtcctccggcccctgaatgcggctaatcccaactgcggagcatacactctcaagccagagggtagtgtgtcgtaatgggcaactctgcagcggaaccgactactttgggtgtccgtgtttcattttattcctatactggctgcttatggtgacaattgagagattgttaccatatagctattggattggccatccggtgactaacagagctattatatatctttttgttgggtttataccacttagcttgaaagaggttaaaactctacattacattttaatactgaacaccgcaaa

SEQ ID NO: 81 - RNA, 737 nt, synthetic construct
  misc_feature 1..737: note = sequence of IRES element
  source 1..737: mol_type = other RNA
ttaaaacagcctgtgggttgatcccacccacagggcccattgggcgctagcactctggtatcacggtacccttgtgcgcctgttttatgtcccttccctcaactgtaacttagaagtaacgcacaccgatcaacagtcagcgtggcacaccagccatgttttgatcaagcacttctgttaccccggaccgagtatcaacagactgctcacgcggttgaaggagaaagtgttcgttatccggccaactacttcgaaaaacctagtaacaccatggaagttgcagagtgtttcgctcagcactaccccagtgtagatcaggtcgatgagtcaccgcatcccccacgggcgaccgtggcggtggctgcgttggcggcctgcctatgggggaacccataggacgctctaatacagacatggtgcgaagagtccattgagctagttggtagtcctccggcccctgaatgcggctaatcctaactgcggagcacacaccttcaagccagagggcagtgtgtcgtaacgggcaactctgcagcggaaccgactactttgggtgtccgtgtttcattttattcttatactggctgcttatggtgacaattgagagattgttaccatatagctattggattggccatccagtgactagcagagctattatatacctctttgttgggtttataccacctaatttgaaagaagttaaaacattagaattcattattaaattgaataca

SEQ ID NO: 82 - RNA, 683 nt, synthetic construct
  misc_feature 1..683: note = sequence of IRES element
  source 1..683: mol_type = other RNA
ttaaaacagcctgtgggttgcacccacccacagggcccacagggcgctagcactctggtatcacggtacctttgtgcgcctgttttattaccccttccccaattgaaaattagaagcaatgcacaccgatcaacagcaggcgtggcgcaccagtcacgtctcgatcaagcacttctgtttccccggaccgagtatcaatagactgctcacgcggttgaaggagaaagtgttcgttatccggctaaccacttcgagaaacccagtaacaccatgaaagttgcagggtgtttcgctcagcacttccccagtgtagatcaggtcgatgagtcaccgcgttccccacgggcgaccgtggcggtggctgcgttggcggcctgcctatgggttaacccataggacgctctaatacagacatggtgcgaagagtttattgagctggttagtatctcctccggcccctgaatgcggctaatcctaactgcggagcacacaccctcaagccagagggcagtgtgtcgtaacgggcaactctgcagcggaaccgactactttgggtgtccgtgtttccttttattcttatactggctgcttatggtgacaatcgaggaattgttaccatatagctattggattggccatccggtgtctaacagagcgattatatacctctttgttggatttat

SEQ ID NO: 83 - RNA, 742 nt, synthetic construct
  misc_feature 1..742: note = sequence of IRES element
  source 1..742: mol_type = other RNA
ttaaaacagcctgtgggttgatcccacccacagggcccactgggcgctagcactctggtatcacggtacctttgtgcgcctgttttatacttcctcccccaactgcaacttagaagtaacacaaaccgatcaacagtcagcgtggcacaccagccacgttttgatcaaacacttctgttaccccggactgagtatcaatagactgctcacgcggttgaaggagaaaacgttcgttatccggccaactacttcgagaaacctagtaacgccatggaagttgtggagtgtttcgctcagcactaccccagtgtagatcaggttgatgagtcaccgcattccccacgggtgaccgtggcggtggctgcgttggcggcctgcccatggggaaacccatgggacgctcttatacagacatggtgcgaagagtctattgagctagttggtagtcctccggcccctgaatgcggctaatcctaactgcggagcacacaccctcaagccagagggcagtgtgtcgtaacgggcaactctgcagcggaaccgactactttgggtgtccgtgtttcattttattcctatactggctgcttatggtgacaattgagagattgttaccatatagctattggattggccatccggtgactaacagagctattatatatctttttgttgggtttataccacttagcttgaaagaggttaaaactctacattacattttaatactgaacaccgcaaa

SEQ ID NO: 84 - RNA, 737 nt, synthetic construct
  misc_feature 1..737: note = sequence of IRES element
  source 1..737: mol_type = other RNA
ttaaaacagcctgtgggttgatcccacccacagggcccattgggcgctagcactctggtatcacggtacccttgtgcgcctgttttatgtcccttccctcaactgtaacttagaagtaacgcacaccgatcaacagtcagcgtggcacaccagccatgttttgatcaagcacttctgttaccccggaccgagtatcaacagactgctcacgcggttgaaggagaaagtgttcgttatccggccaactacttcgaaaaacctagtaacaccatggaagttgcagagtgtttcgctcagcactaccccagtgtagatcaggtcgatgagtcaccgcatcccccacgggcgaccgtggcggtggctgcgttggcggcctgcctatgggggaacccataggacgctctaatacagacatggtgcgaagagtccattgagctagttggtagtcctccggcccctgaatgcggctaatcctaactgcggagcacacaccctcaagccagagggcagtgtgtcgtaacgggcaactctgcagcggaaccgactactttgggtgtccgtgtttcattttattcttatactggctgcttatggtgacaattgagagattgttaccatatagctattggattggccatccagtgactagcagagctattatatacctctttgttgggtttataccacctaatttgaaagaagttaaaacattagaattcattattaaattgaataca

SEQ ID NO: 85 - RNA, 50 nt, synthetic construct
  misc_feature 1..50: note = sequence of 5spacer region
  source 1..50: mol_type = other RNA
aaaaaacaaaaacaaaaaaaacaaaaaaacaaaaaaaaaaccaaaacaca

SEQ ID NO: 86 - RNA, 50 nt, synthetic construct
  misc_feature 1..50: note = sequence of 5spacer region
  source 1..50: mol_type = other RNA
aaaaacaaaaaacaaaaaaaaaaccaaaaaaacaaaaaaaacaaaacaca

SEQ ID NO: 87 - RNA, 25 nt, synthetic construct
  misc_feature 1..25: note = sequence of 3spacer region
  source 1..25: mol_type = other RNA
aaaaaaacaaaaaaacaaaacaaac

SEQ ID NO: 88 - RNA, 22 nt, synthetic construct
  misc_feature 1..22: note = sequence of 3spacer region
  source 1..22: mol_type = other RNA
aaaaacaaaaaacaaaacaaac

SEQ ID NO: 89 - RNA, 19 nt, synthetic construct
  misc_feature 1..19: note = sequence of 3spacer region
  source 1..19: mol_type = other RNA
aaaaaacaaaaaacaaaac

SEQ ID NO: 90 - DNA, 16 bp, synthetic construct
  misc_feature 1..16: note = sequence of first exon
  source 1..16: mol_type = other DNA
agacgctacggactta

SEQ ID NO: 91 - DNA, 51 bp, synthetic construct
  misc_feature 1..51: note = sequence of second exon
  source 1..51: mol_type = other DNA
aaaatccgttgaccttaaacggtcgtgtgggttcaagtccctccaccccca

SEQ ID NO: 92 - DNA, 114 bp, synthetic construct
  misc_feature 1..114: note = sequence of 5intron
  source 1..114: mol_type = other DNA
aataattgagccttaaagaagaaattctttaagtggatgctctcaaactcagggaaacctaaatctagttatagacaaggcaatcctgagccaagccgaagtagtaattagtaa

SEQ ID NO: 93 - DNA, 131 bp, synthetic construct
  misc_feature 1..131: note = sequence of 3intron
  source 1..131: mol_type = other DNA
aacaatagatgacttacaactaatcggaaggtgcagagactcgacgggagctaccctaacgtcaagacgagggtaaagagagagtccaattctcaaagccaataggcagtagcgaaagctgcaagagaatg

SEQ ID NO: 94 - DNA, 21 bp, synthetic construct
  misc_feature 1..21: note = sequence of 5homologous arm
  source 1..21: mol_type = other DNA
accgtcagttgctcactgtgc

SEQ ID NO: 95 - DNA, 21 bp, synthetic construct
  misc_feature 1..21: note = sequence of 5homologous arm
  source 1..21: mol_type = other DNA
accgtgctatgtccacgtgtc

SEQ ID NO: 96 - DNA, 21 bp, synthetic construct
  misc_feature 1..21: note = sequence of 3homologous arm
  source 1..21: mol_type = other DNA
gcacagtgagcaactgacgga

SEQ ID NO: 97 - DNA, 21 bp, synthetic construct
  misc_feature 1..21: note = sequence of 3homologous arm
  source 1..21: mol_type = other DNA
gacacgtggacatagcacgga